European Patent Specification EP 3 752 128 B1, published January 15, 2025. Title: Nukleinsäure-basiertes Botolinum Neurotoxin zur therapeutischen Anwendung. Applicant: Füner, Jonas. The sequence listing filed with the application follows.

SEQUENCE LISTING (6 sequences)

SEQ ID NO: 1 - protein, 1296 aa, Clostridium botulinum
MPFVNKQFNYKDPVNGVDIAYIKIPNAGQMQPVKAFKIHNKIWVIPERDTFTNPEEGDLNPPPEAKQVPVSYYDSTYLSTDNEKDNYLKGVTKLFERIYSTDLGRMLLTSIVRGIPFWGGSTIDTELKVIDTNCINVIQPDGSYRSEELNLVIIGPSADIIQFECKSFGHEVLNLTRNGYGSTQYIRFSPDFTFGFEESLEVDTNPLLGAGKFATDPAVTLAHELIHAGHRLYGIAINPNRVFKVNTNAYYEMSGLEVSFEELRTFGGHDAKFIDSLQENEFRLYYYNKFKDIASTLNKAKSIVGTTASLQYMKNVFKEKYLLSEDTSGKFSVDKLKFDKLYKMLTEIYTEDNFVKFFKVLNRKTYLNFDKAVFKINIVPKVNYTIYDGFNLRNTNLAANFNGQNTEINNMNFTKLKNFTGLFEFYKLLCVRGIITSKTKSLDKGYNKALNDLCIKVNNWDLFFSPSEDNFTNDLNKGEEITSDTNIEAAEENISLDLIQQYYLTFNFDNEPENISIENLSSDIIGQLELMPNIERFPNGKKYELDKYTMFHYLRAQEFEHGKSRIALTNSVNEALLNPSRVYTFFSSDYVKKVNKATEAAMFLGWVEQLVYDFTDETSEVSTTDKIADITIIIPYIGPALNIGNMLYKDDFVGALIFSGAVILLEFIPEIAIPVLGTFALVSYIANKVLTVQTIDNALSKRNEKWDEVYKYIVTNWLAKVNTQIDLIRKKMKEALENQAEATKAIINYQYNQYTEEEKNNINFNIDDLSSKLNESINKAMININKFLNQCSVSYLMNSMIPYGVKRLEDFDASLKDALLKYIYDNRGTLIGQVDRLKDKVNNTLSTDIPFQLSKYVDNQRLLSTFTEYIKNIINTSILNLRYESNHLIDLSRYASKINIGSKVNFDPIDKNQIQLFNLESSKIEVILKNAIVYNSMYENFSTSFWIRIPKYFNSISLNNEYTIINCMENNSGWKVSLNYGEIIWTLQDTQEIKQRVVFKYSQMINISDYINRWIFVTITNNRLNNSKIYINGRLIDQKPISNLGNIHASNNIMFKLDGCRDTHRYIWIKYFNLFDKELNEKEIKDLYDNQSNSGILKDFWGDYLQYDKPYYMLNLYDPNKYVDVNNVGIRGYMYLKGPRGSVMTTNIYLNSSLYRGTKFIIKKYASGNKDNIVRNNDRVYINVVVKNKEYRLATNASQAGVEKILSALEIPDVGNLSQVVVMKSKNDQGITNKCKMNLQDNNGNDIGFIGFHQFNNIAKLVASNWYNRQIERSSRTLGCSWEFIPVDDGWGERPL

SEQ ID NO: 2 - protein, 1252 aa, Clostridium botulinum
MPKINSFNYNDPVNDKTILYIKPGGCQQFYKSFNIMKNIWIIPERNVIGTIPQDFLPPTSLKNGDSSYYDPNYLQSNEEKDRFLKIVTKIFNRINDNLSGRILLEELSKANPYLGNDNTPDNQFHIGDASAVEIKFSNGNQSILLPNVIIMGAEPDLFETNSSNISLRNNYMPSNHGFGSIAIVTFSPEYSFRFNDNSMNEFIQDPALTLMHELIHSLHGLYGAKRITTKYTITQQQNPLITNIRGTNIEEFLTFGGTDLNIITSAQYNDIYTNLLADYKKIASKLSKVQVSNPQLNPYKDIFQEKYGLDKNASGIYSVNINKFDDIFKKLYSFTEFDLATKFQVKCRQTYIGQYKYFKLSNLLNNSIYNISEGYNINTLKVNFRGQNTNLNPRIITQLTGRGLVKKIIRFCKNIVFSKGITKSICIEINNGELFFVASENSYNDDNINTPKEIDDTVTSNNNYENDLDQVILNFNSESAPGLSDEKLNLTIQNDAYIPKYDSNGTSDIEQHDVNELNVFFYLDAQKVPEGENNVNLTSSIDTALLEQPKIYTFFSSEFINNVNKPVQAALFVSWIQQVLVDFTTEANQKSTVDKIADISIVVPYIGLALNIGNEAQKGNFKDALELLGAGILLEFEPELLIPTILVFTIKSFLGSSDNKNKVIKAINNALKERDEKWKEVYSFIVSNWMTKINTQFNKRKEQMYQALQNQVNAIKTIIESKYNSYTLEEKNELTNKYDIKQIENELNQKVSIAMNNIDRFLTESSISYLMKLINEVKINKLREYDENVKTYLLNYIIQHGSILGESQQELNSMVTDTLNNSIPFKLSSYTDDKILISYFNKFFKRIKSSSVLNMRYKNDKYVDTSGYDSNININGDVYKYPTNKNQFGIYNDKLSEVNISQNDYIIYDNKYKNFSISFWVRIPNYDNKIVNVNNEYTIINCMRDNNSGWKVSLNHNEIIWTLQDNAGINQKLAFNYGNANGISDYINKWIFVTITNDRLGDSKLYINGNLIDQKSILNLGNIHVSDNILFKIVNCSYTRYIGIRYFNIFDKELDETEIQTLYSNEPNTNILKDFWGNYLLYDKEYYLLNVLKPNNFIDRRKDSTLSINNIRSTILLANRLYSGIKVKIQRVNNSSTNDNLVRKNDQVYINFVASKTHLFPLYADTATTNKEKTIKISSSGNRFNQVVVMNSVGNNCTMNFKNNNGNNIGLLGFKADTVVASTWYYTHMRDHTNSNGCFWNFISEEHGWQEK

SEQ ID NO: 3 - protein, 1291 aa, Clostridium botulinum
MPVTINNFNYNDPIDNDNIIMMEPPFARGTGRYYKAFKITDRIWIIPERYTFGYKPEDFNKSSGIFNRDVCEYYDPDYLNTNDKKNIFFQTLIKLFNRIKSKPLGEKLLEMIINGIPYLGDRRVPLEEFNTNIASVTVNKLISNPGEVERKKGIFANLIIFGPGPVLNENETIDIGIQNHFASREGFGGIMQMKFCPEYVSVFNNVQENKGASIFNRRGYFSDPALILMHELIHVLHGLYGIKVDDLPIVPNEKKFFMQSTDTIQAEELYTFGGQDPSIISPSTDKSIYDKVLQNFRGIVDRLNKVLVCISDPNININIYKNKFKDKYKFVEDSEGKYSIDVESFNKLYKSLMLGFTEINIAENYKIKTRASYFSDSLPPVKIKNLLDNEIYTIEEGFNISDKNMGKEYRGQNKAINKQAYEEISKEHLAVYKIQMCKSVKVPGICIDVDNENLFFIADKNSFSDDLSKNERVEYNTQNNYIGNDFPINELILDTDLISKIELPSENTESLTDFNVDVPVYEKQPAIKKVFTDENTIFQYLYSQTFPLNIRDISLTSSFDDALLVSSKVYSFFSMDYIKTANKVVEAGLFAGWVKQIVDDFVIEANKSSTMDKIADISLIVPYIGLALNVGDETAKGNFESAFEIAGSSILLEFIPELLIPVVGVFLLESYIDNKNKIIKTIDNALTKRVEKWIDMYGLIVAQWLSTVNTQFYTIKEGMYKALNYQAQALEEIIKYKYNIYSEEEKSNININFNDINSKLNDGINQAMDNINDFINECSVSYLMKKMIPLAVKKLLDFDNTLKKNLLNYIDENKLYLIGSVEDEKSKVDKYLKTIIPFDLSTYSNIEILIKIFNKYNSEILNNIILNLRYRDNNLIDLSGYGAKVEVYDGVKLNDKNQFKLTSSADSKIRVTQNQNIIFNSMFLDFSVSFWIRIPKYRNDDIQNYIHNEYTIINCMKNNSGWKISIRGNRIIWTLIDINGKTKSVFFEYNIREDISEYINRWFFVTITNNLDNAKIYINGTLESNMDIKDIGEVIVNGEITFKLDGDVDRTQFIWMKYFSIFNTQLNQSNIKEIYKIQSYSEYLKDFWGNPLMYNKEYYMFNAGNKNSYIKLVKDSSVGEILIRSKYNQNSNYINYRNLYIGEKFIIRRESNSQSINDDIVRKEDYIHLDLVLHHEEWRVYAYKYFKEQEEKLFLSIISDSNEFYKTIEIKEYDEQPSYSCQLLFKKDEESTDDIGLIGIHRFYESGVLRKKYKDYFCISKWYLKEVKRKPYKSNLGCNWQFIPKDEGWTE

SEQ ID NO: 4 - protein, 1296 aa, Artificial Sequence
  BoNT/A1 mit Proteasesplatsignal
MPFVNKQFNYKDPVNGVDIAYIKIPNAGQMQPVKAFKIHNKIWVIPERDTFTNPEEGDLNPPPEAKQVPVSYYDSTYLSTDNEKDNYLKGVTKLFERIYSTDLGRMLLTSIVRGIPFWGGSTIDTELKVIDTNCINVIQPDGSYRSEELNLVIIGPSADIIQFECKSFGHEVLNLTRNGYGSTQYIRFSPDFTFGFEESLEVDTNPLLGAGKFATDPAVTLAHELIHAGHRLYGIAINPNRVFKVNTNAYYEMSGLEVSFEELRTFGGHDAKFIDSLQENEFRLYYYNKFKDIASTLNKAKSIVGTTASLQYMKNVFKEKYLLSEDTSGKFSVDKLKFDKLYKMLTEIYTEDNFVKFFKVLNRKTYLNFDKAVFKINIVPKVNYTIYDGFNLRNTNLAANFNGQNTEINNMNFTKLKNFTGLFEFYKLLCVRGIITSKTKSLVPRGSKALNDLCIKVNNWDLFFSPSEDNFTNDLNKGEEITSDTNIEAAEENISLDLIQQYYLTFNFDNEPENISIENLSSDIIGQLELMPNIERFPNGKKYELDKYTMFHYLRAQEFEHGKSRIALTNSVNEALLNPSRVYTFFSSDYVKKVNKATEAAMFLGWVEQLVYDFTDETSEVSTTDKIADITIIIPYIGPALNIGNMLYKDDFVGALIFSGAVILLEFIPEIAIPVLGTFALVSYIANKVLTVQTIDNALSKRNEKWDEVYKYIVTNWLAKVNTQIDLIRKKMKEALENQAEATKAIINYQYNQYTEEEKNNINFNIDDLSSKLNESINKAMININKFLNQCSVSYLMNSMIPYGVKRLEDFDASLKDALLKYIYDNRGTLIGQVDRLKDKVNNTLSTDIPFQLSKYVDNQRLLSTFTEYIKNIINTSILNLRYESNHLIDLSRYASKINIGSKVNFDPIDKNQIQLFNLESSKIEVILKNAIVYNSMYENFSTSFWIRIPKYFNSISLNNEYTIINCMENNSGWKVSLNYGEIIWTLQDTQEIKQRVVFKYSQMINISDYINRWIFVTITNNRLNNSKIYINGRLIDQKPISNLGNIHASNNIMFKLDGCRDTHRYIWIKYFNLFDKELNEKEIKDLYDNQSNSGILKDFWGDYLQYDKPYYMLNLYDPNKYVDVNNVGIRGYMYLKGPRGSVMTTNIYLNSSLYRGTKFIIKKYASGNKDNIVRNNDRVYINVVVKNKEYRLATNASQAGVEKILSALEIPDVGNLSQVVVMKSKNDQGITNKCKMNLQDNNGNDIGFIGFHQFNNIAKLVASNWYNRQIERSSRTLGCSWEFIPVDDGWGERPL

SEQ ID NO: 5 - DNA, 3888 bp, Artificial Sequence
  Codon optimierte DNA-Sequenz für die Expression in humanen Zellen
atgcccttcgtgaacaagcagttcaactacaaggaccccgtgaacggcgtggacatcgcctacatcaagatccccaacgccggccagatgcagcccgtgaaggccttcaagatccacaacaagatctgggtgatccccgagcgcgacaccttcaccaaccccgaggagggcgacctgaaccccccccccgaggccaagcaggtgcccgtgagctactacgacagcacctacctgagcaccgacaacgagaaggacaactacctgaagggcgtgaccaagctgttcgagcgcatctacagcaccgacctgggccgcatgctgctgaccagcatcgtgcgcggcatccccttctggggcggcagcaccatcgacaccgagctgaaggtgatcgacaccaactgcatcaacgtgatccagcccgacggcagctaccgcagcgaggagctgaacctggtgatcatcggccccagcgccgacatcatccagttcgagtgcaagagcttcggccacgaggtgctgaacctgacccgcaacggctacggcagcacccagtacatccgcttcagccccgacttcaccttcggcttcgaggagagcctggaggtggacaccaaccccctgctgggcgccggcaagttcgccaccgaccccgccgtgaccctggcccacgagctgatccacgccggccaccgcctgtacggcatcgccatcaaccccaaccgcgtgttcaaggtgaacaccaacgcctactacgagatgagcggcctggaggtgagcttcgaggagctgcgcaccttcggcggccacgacgccaagttcatcgacagcctgcaggagaacgagttccgcctgtactactacaacaagttcaaggacatcgccagcaccctgaacaaggccaagagcatcgtgggcaccaccgccagcctgcagtacatgaagaacgtgttcaaggagaagtacctgctgagcgaggacaccagcggcaagttcagcgtggacaagctgaagttcgacaagctgtacaagatgctgaccgagatctacaccgaggacaacttcgtgaagttcttcaaggtgctgaaccgcaagacctacctgaacttcgacaaggccgtgttcaagatcaacatcgtgcccaaggtgaactacaccatctacgacggcttcaacctgcgcaacaccaacctggccgccaacttcaacggccagaacaccgagatcaacaacatgaacttcaccaagctgaagaacttcaccggcctgttcgagttctacaagctgctgtgcgtgcgcggcatcatcaccagcaagaccaagagcctggacaagggctacaacaaggccctgaacgacctgtgcatcaaggtgaacaactgggacctgttcttcagccccagcgaggacaacttcaccaacgacctgaacaagggcgaggagatcaccagcgacaccaacatcgaggccgccgaggagaacatcagcctggacctgatccagcagtactacctgaccttcaacttcgacaacgagcccgagaacatcagcatcgagaacctgagcagcgacatcatcggccagctggagctgatgcccaacatcgagcgcttccccaacggcaagaagtacgagctggacaagtacaccatgttccactacctgcgcgcccaggagttcgagcacggcaagagccgcatcgccctgaccaacagcgtgaacgaggccctgctgaaccccagccgcgtgtacaccttcttcagcagcgactacgtgaagaaggtgaacaaggccaccgaggccgccatgttcctgggctgggtggagcagctggtgtacgacttcaccgacgagaccagcgaggtgagcaccaccgacaagatcgccgacatcaccatcatcatcccctacatcggccccgccctgaacatcggcaacatgctgtacaaggacgacttcgtgggcgccctgatcttcagcggcgccgtgatcctgctggagttcatccccgagatcgccatccccgtgctgggcaccttcgccctggtgagctacatcgccaacaaggtgctgaccgtgcagaccatcgacaacgccctgagcaagcgcaacgagaagtgggacgaggtgtacaagtacatcgtgaccaactggctggccaaggtgaacacccagatcgacctgatccgcaagaagatgaaggaggccctggagaaccaggccgaggccaccaaggccatcatcaactaccagtacaaccagtacaccgaggaggagaagaacaacatcaacttcaacatcgacgacctgagcagcaagctgaacgagagcatcaacaaggccatgatcaacatcaacaagttcctgaaccagtgcagcgtgagctacctgatgaacagcatgatcccctacggcgtgaagcgcctggaggacttcgacgccagcctgaaggacgccctgctgaagtacatctacgacaaccgcggcaccctgatcggccaggtggaccgcctgaaggacaaggtgaacaacaccctgagcaccgacatccccttccagctgagcaagtacgtggacaaccagcgcctgctgagcaccttcaccgagtacatcaagaacatcatcaacaccagcatcctgaacctgcgctacgagagcaaccacctgatcgacctgagccgctacgccagcaagatcaacatcggcagcaaggtgaacttcgaccccatcgacaagaaccagatccagctgttcaacctggagagcagcaagatcgaggtgatcctgaagaacgccatcgtgtacaacagcatgtacgagaacttcagcaccagcttctggatccgcatccccaagtacttcaacagcatcagcctgaacaacgagtacaccatcatcaactgcatggagaacaacagcggctggaaggtgagcctgaactacggcgagatcatctggaccctgcaggacacccaggagatcaagcagcgcgtggtgttcaagtacagccagatgatcaacatcagcgactacatcaaccgctggatcttcgtgaccatcaccaacaaccgcctgaacaacagcaagatctacatcaacggccgcctgatcgaccagaagcccatcagcaacctgggcaacatccacgccagcaacaacatcatgttcaagctggacggctgccgcgacacccaccgctacatctggatcaagtacttcaacctgttcgacaaggagctgaacgagaaggagatcaaggacctgtacgacaaccagagcaacagcggcatcctgaaggacttctggggcgactacctgcagtacgacaagccctactacatgctgaacctgtacgaccccaacaagtacgtggacgtgaacaacgtgggcatccgcggctacatgtacctgaagggcccccgcggcagcgtgatgaccaccaacatctacctgaacagcagcctgtaccgcggcaccaagttcatcatcaagaagtacgccagcggcaacaaggacaacatcgtgcgcaacaacgaccgcgtgtacatcaacgtggtggtgaagaacaaggagtaccgcctggccaccaacgccagccaggccggcgtggagaagatcctgagcgccctggagatccccgacgtgggcaacctgagccaggtggtggtgatgaagagcaagaacgaccagggcatcaccaacaagtgcaagatgaacctgcaggacaacaacggcaacgacatcggcttcatcggcttccaccagttcaacaacatcgccaagctggtggccagcaactggtacaaccgccagatcgagcgcagcagccgcaccctgggctgcagctgggagttcatccccgtggacgacggctggggcgagcgccccctg

SEQ ID NO: 6 - DNA, 63 bp, Artificial Sequence
  Sekretorisches Signal von murinem IgG (Kappa)
atggagaccgacaccctgctgctgtgggtgctgctgctgtgggtgcccggcagcaccggcgac